European Patent Specification EP 3 740 569 B1, published July 26, 2023. Title: Regulatory T cell expressing a chimeric antigen receptor. Applicant: Miltenyi Biotec GmbH. The sequence listing filed with the application follows.

SEQUENCE LISTING (2 sequences)

SEQ ID NO: 1 - protein, 117 aa, Artificial sequence
  anti-dextran VH
EVQLQQSGPELVKPGASVKISCKASGYTFTDYYMNWVKQSHGKSLEWIGDINPNNGGTSYNQKFKGKATLTVDKSSSTAYMELRSLTSEDSAVYYCAPYYYTSSIVWGTGTTVTVSA

SEQ ID NO: 2 - protein, 106 aa, Artificial sequence
  anti-dextran VL
QIVLTQSPAIMSASPGEKVTMTCSASSSVSYMHWYQQKSGTSPKRWIYDTSKLASGVPARFSGSGSGTSYSLTISSMEAEDAATYYCQQWSSNPLTFGAGTKLELK